European Patent Application EP 4 792 833 A1, published August 19, 2026. Title: 一种用于前药给药系统的可裂解连接体化合物及其制备和应用. Applicant: 华东师范大学. Application CN. The sequence listing filed with the application follows.

SEQUENCE LISTING (8 sequences)

SEQ ID NO: 1 - protein, 448 aa, synthetic construct
EVQLVESGGGLVKPGGSLRLSCAASGFTFSSYAVSWVRQAPGKGLEWVASISGGGIYIYYPDSVKGRFTISRDNAKNSLYLQMNSLRAEDTAVYYCARHGGAGYFDYWGQGTLVTVSSASTKGPSVFPLAPSSKSTSGGTAALGCLVKDYFPEPVTVSWNSGALTSGVHTFPAVLQSSGLYSLSSVVTVPSSSLGTQTYICNVNHKPSNTKVDKKVEPKSCDKTHTCPPCPAPELLGGPSVFLFPPKPKDTLMISRTPEVTCVVVDVSHEDPEVKFNWYVDGVEVHNAKTKPREEQYNSTYRVVSVLTVLHQDWLNGKEYKCKVSNKALPAPIEKTISKAKGQPREPQVYTLPPSRDELTKNQVSLTCLVKGFYPSDIAVEWESNGQPENNYKTTPPVLDSDGSFFLYSKLTVDKSRWQQGNVFSCSVMHEALHNHYTQKSLSLSPGK

SEQ ID NO: 2 - protein, 215 aa, synthetic construct
DSQMTQSPSSLSASVGDRVTITCRGSESVHSYLAWYQQKPGKAPKLLVYNAKTLQSGVPSRFSGSGSGTDFTLTISSLQPEDFATYYCQQHYGSPPWTFGGGTKVEIKRTVAAPSVFIFPPSDEQLKSGTASVVCLLNNFYPREAKVQWKVDNALQSGNSQESVTEQDSKDSTYSLSSTLTLSKADYEKHKVYACEVTHQGLSSPVTKSFNRGEC

SEQ ID NO: 3 - protein, 450 aa, synthetic construct
EVQLVESGGGLVQPGGSLRLSCAASGFNIKDTYIHWVRQAPGKGLEWVARIYPTNGYTRYADSVKGRFTISADTSKNTAYLQMNSLRAEDTAVYYCSRWGGDGFYAMDYWGQGTLVTVSSASTKGPSVFPLAPSSKSTSGGTAALGCLVKDYFPEPVTVSWNSGALTSGVHTFPAVLQSSGLYSLSSVVTVPSSSLGTQTYICNVNHKPSNTKVDKKVEPKSCDKTHTCPPCPAPELLGGPSVFLFPPKPKDTLMISRTPEVTCVVVDVSHEDPEVKFNWYVDGVEVHNAKTKPREEQYNSTYRVVSVLTVLHQDWLNGKEYKCKVSNKALPAPIEKTISKAKGQPREPQVYTLPPSREEMTKNQVSLTCLVKGFYPSDIAVEWESNGQPENNYKTTPPVLDSDGSFFLYSKLTVDKSRWQQGNVFSCSVMHEALHNHYTQKSLSLSPGK

SEQ ID NO: 4 - protein, 214 aa, synthetic construct
DIQMTQSPSSLSASVGDRVTITCRASQDVNTAVAWYQQKPGKAPKLLIYSASFLYSGVPSRFSGSRSGTDFTLTISSLQPEDFATYYCQQHYTTPPTFGQGTKVEIKRTVAAPSVFIFPPSDEQLKSGTASVVCLLNNFYPREAKVQWKVDNALQSGNSQESVTEQDSKDSTYSLSSTLTLSKADYEKHKVYACEVTHQGLSSPVTKSFNRGEC

SEQ ID NO: 5 - protein, 450 aa, synthetic construct
EVQLVQSGSELKKPGASVKVSCKASGYTFTNYGMNWVRQAPGQGLEYMGWINTYTGEPTYGEDFKGRFVFSLDTSVSTAYLQISSLKAEDTAVYYCAKKGDSTVVDFDVWGQGTTVTVSSASTKGPSVFPLAPSSKSTSGGTAALGCLVKDYFPEPVTVSWNSGALTSGVHTFPAVLQSSGLYSLSSVVTVPSSSLGTQTYICNVNHKPSNTKVDKKVEPKSCDKTHTCPPCPAPELLGGPSVFLFPPKPKDTLMISRTPEVTCVVVDVSHEDPEVKFNWYVDGVEVHNAKTKPREEQYNSTYRVVSVLTVLHQDWLNGKEYKCKVSNKALPAPIEKTISKAKGQPREPQVYTLPPSRDELTKNQVSLTCLVKGFYPSDIAVEWESNGQPENNYKTTPPVLDSDGSFFLYSKLTVDKSRWQQGNVFSCSVMHEALHNHYTQKSLSLSPGK

SEQ ID NO: 6 - protein, 218 aa, synthetic construct
DIVLTQSPDSLAVSLGERATINCKASQSVDYDGDSYMNWYQQKPGQPPKLLIYAASILESGIPDRFSGSGSGTDFTLTISSLQAEDVAVYYCQQSYEDPLTFGQGTKLEIKRTVAAPSVFIFPPSDEQLKSGTASVVCLLNNFYPREAKVQWKVDNALQSGNSQESVTEQDSKDSTYSLSSTLTLSKADYEKHKVYACEVTHQGLSSPVTKSFNRGEC

SEQ ID NO: 7 - protein, 450 aa, synthetic construct
QVQLVESGGGLVKPGGSLRLSCAASGFTFSDYYMSWIRQAPGKGLEWVSYITYSGSTIYYADSVKGRFTISRDNAKSSLYLQMNSLRAEDTAVYYCARDRGTTMVPFDYWGQGTLVTVSSASTKGPSVFPLAPSSKSTSGGTAALGCLVKDYFPEPVTVSWNSGALTSGVHTFPAVLQSSGLYSLSSVVTVPSSSLGTQTYICNVNHKPSNTKVDKKVEPKSCDKTHTCPPCPAPELLGGPSVFLFPPKPKDTLMISRTPEVTCVVVDVSHEDPEVKFNWYVDGVEVHNAKTKPREEQYNSTYRVVSVLTVLHQDWLNGKEYKCKVSNKALPAPIEKTISKAKGQPREPQVYTLPPSRDELTKNQVSLTCLVKGFYPSDIAVEWESNGQPENNYKTTPPVLDSDGSFFLYSKLTVDKSRWQQGNVFSCSVMHEALHNHYTQKSLSLSPGK

SEQ ID NO: 8 - protein, 214 aa, synthetic construct
DIQMTQSPSSLSASVGDRVTITCQASQDITNYLNWYQQKPGKAPKLLIYAASNLETGVPSRFSGSGSGTDFTFTISGLQPEDIATYYCQQYDNLPLTFGGGTKVEIKRTVAAPSVFIFPPSDEQLKSGTASVVCLLNNFYPREAKVQWKVDNALQSGNSQESVTEQDSKDSTYSLSSTLTLSKADYEKHKVYACEVTHQGLSSPVTKSFNRGEC